European Patent Application EP 4 729 541 A1, published April 22, 2026. Title: ANTI- IGFBP7 ANTIBODIES AND USES THEREOF. Applicant: Paolo Fiorina. The sequence listing filed with the application follows.

SEQUENCE LISTING (128 sequences)

SEQ ID NO: 1 - protein, 5 aa, synthetic construct
DYAMH

SEQ ID NO: 2 - protein, 17 aa, synthetic construct
GISWNSGSIGYADSVKG

SEQ ID NO: 3 - protein, 11 aa, synthetic construct
ANYYDSSALDY

SEQ ID NO: 4 - protein, 12 aa, synthetic construct
DISGSQLVLLDY

SEQ ID NO: 5 - protein, 13 aa, synthetic construct
DIWATVTPAAFDY

SEQ ID NO: 6 - protein, 11 aa, synthetic construct
DNSGSGRYFDY

SEQ ID NO: 7 - protein, 12 aa, synthetic construct
DVTAMDTVGFQH

SEQ ID NO: 8 - protein, 13 aa, synthetic construct
GLVAATTPPYFDY

SEQ ID NO: 9 - protein, 5 aa, synthetic construct
SYAIS

SEQ ID NO: 10 - protein, 17 aa, synthetic construct
GIIPIFGTANYAQKFQG

SEQ ID NO: 11 - protein, 13 aa, synthetic construct
GTYYYDSSGTPDY

SEQ ID NO: 12 - protein, 16 aa, synthetic construct
PSVLEWTYYYYYGMDV

SEQ ID NO: 13 - protein, 17 aa, synthetic construct
RIIPIFGIANYAQKFQG

SEQ ID NO: 14 - protein, 5 aa, synthetic construct
SYAMH

SEQ ID NO: 15 - protein, 17 aa, synthetic construct
AISSNGGSTYYADSVKG

SEQ ID NO: 16 - protein, 12 aa, synthetic construct
GEQWLAYNWFDP

SEQ ID NO: 17 - protein, 17 aa, synthetic construct
VISYDGSNKYYADSVKG

SEQ ID NO: 18 - protein, 12 aa, synthetic construct
DSGPTTVTTFDY

SEQ ID NO: 19 - protein, 10 aa, synthetic construct
SVGYLNWFDP

SEQ ID NO: 20 - protein, 5 aa, synthetic construct
SYAMS

SEQ ID NO: 21 - protein, 17 aa, synthetic construct
AISGSGGSTYYADSVKG

SEQ ID NO: 22 - protein, 16 aa, synthetic construct
DHPPSVYSSSWLRFDY

SEQ ID NO: 23 - protein, 19 aa, synthetic construct
DLFLDLYDSSGYYLVPQIH

SEQ ID NO: 24 - protein, 5 aa, synthetic construct
SYGMH

SEQ ID NO: 25 - protein, 12 aa, synthetic construct
HGDYGGYQYFQH

SEQ ID NO: 26 - protein, 5 aa, synthetic construct
SYSMN

SEQ ID NO: 27 - protein, 17 aa, synthetic construct
SISSSSSYIYYADSVKG

SEQ ID NO: 28 - protein, 14 aa, synthetic construct
DRDTYYDYGDNFDY

SEQ ID NO: 29 - protein, 5 aa, synthetic construct
SYSMS

SEQ ID NO: 30 - protein, 16 aa, synthetic construct
AISGSGGTYYADSVKG

SEQ ID NO: 31 - protein, 7 aa, synthetic construct
SLRAFSY

SEQ ID NO: 32 - protein, 5 aa, synthetic construct
SYWIG

SEQ ID NO: 33 - protein, 17 aa, synthetic construct
IIYPGDSDTRYSPSFQG

SEQ ID NO: 34 - protein, 14 aa, synthetic construct
LGVSGSYRRSGMDV

SEQ ID NO: 35 - protein, 14 aa, synthetic construct
TGTSSDVGGYNYVS

SEQ ID NO: 36 - protein, 7 aa, synthetic construct
DVSNRPS

SEQ ID NO: 37 - protein, 10 aa, synthetic construct
SSYTSSSTWV

SEQ ID NO: 38 - protein, 14 aa, synthetic construct
TGSSSNIGAGYDVH

SEQ ID NO: 39 - protein, 7 aa, synthetic construct
GNSNRPS

SEQ ID NO: 40 - protein, 10 aa, synthetic construct
QSYDSSLSVV

SEQ ID NO: 41 - protein, 16 aa, synthetic construct
RSSQSLLHSNGYNYLD

SEQ ID NO: 42 - protein, 7 aa, synthetic construct
LGSNRAS

SEQ ID NO: 43 - protein, 8 aa, synthetic construct
MQALQTPL

SEQ ID NO: 44 - protein, 11 aa, synthetic construct
SSYTSSSTLVV

SEQ ID NO: 45 - protein, 9 aa, synthetic construct
MQALQTPYT

SEQ ID NO: 46 - protein, 10 aa, synthetic construct
SSYTSSSTLV

SEQ ID NO: 47 - protein, 13 aa, synthetic construct
SGSSSNIGNNYVS

SEQ ID NO: 48 - protein, 7 aa, synthetic construct
DNNKRPS

SEQ ID NO: 49 - protein, 11 aa, synthetic construct
GTWDSSLSAVV

SEQ ID NO: 50 - protein, 11 aa, synthetic construct
QASQDISNYLN

SEQ ID NO: 51 - protein, 7 aa, synthetic construct
DASNLET

SEQ ID NO: 52 - protein, 9 aa, synthetic construct
QQYDNLPLT

SEQ ID NO: 53 - protein, 13 aa, synthetic construct
SGSSSNIGSNTVN

SEQ ID NO: 54 - protein, 7 aa, synthetic construct
SNNQRPS

SEQ ID NO: 55 - protein, 11 aa, synthetic construct
AAWDDSLNGYV

SEQ ID NO: 56 - protein, 12 aa, synthetic construct
QSYDSSLSGWGV

SEQ ID NO: 57 - protein, 13 aa, synthetic construct
SGSSSNIGSNYVY

SEQ ID NO: 58 - protein, 7 aa, synthetic construct
RNSQRPS

SEQ ID NO: 59 - protein, 12 aa, synthetic construct
AAWDDSLSVPYV

SEQ ID NO: 60 - protein, 11 aa, synthetic construct
RASQSISSWLA

SEQ ID NO: 61 - protein, 7 aa, synthetic construct
KASSLES

SEQ ID NO: 62 - protein, 9 aa, synthetic construct
QQYNSYLIT

SEQ ID NO: 63 - protein, 12 aa, synthetic construct
QSYDSSLSGFVV

SEQ ID NO: 64 - protein, 10 aa, synthetic construct
SSYTSSSTVV

SEQ ID NO: 65 - protein, 12 aa, synthetic construct
QSYDSSLSGSWV

SEQ ID NO: 66 - protein, 11 aa, synthetic construct
SGDALPKQYAY

SEQ ID NO: 67 - protein, 7 aa, synthetic construct
KDSERPS

SEQ ID NO: 68 - protein, 11 aa, synthetic construct
QSADSSGTYYV

SEQ ID NO: 69 - protein, 9 aa, synthetic construct
MQSLRTPLT

SEQ ID NO: 70 - protein, 12 aa, synthetic construct
RASQSVSSSYLA

SEQ ID NO: 71 - protein, 7 aa, synthetic construct
GASSRAT

SEQ ID NO: 72 - protein, 9 aa, synthetic construct
QQYGSSPLT

SEQ ID NO: 73 - protein, 120 aa, synthetic construct
EVQLLESGGGLVQPGRSLRLSCAATGFTFDDYAMHWVRQAPGKGLEWVSGISWNSGSIGYADSVKGRFTISRDNAKNSLYLQMNSLRAEDTALYYCAKANYYDSSALDYWGQGTLVTVSS

SEQ ID NO: 74 - protein, 121 aa, synthetic construct
QVQLVQSGGGLVQPGRSLRLSCAASGFTFDDYAMHWVRQAPGKGLEWVSGISWNSGSIGYADSVKGRFTISRDNAKNSLYLQMNSLRAEDTALYYCAKDISGSQLVLLDYWGQGTTVTVSS

SEQ ID NO: 75 - protein, 122 aa, synthetic construct
QVQLVQSGGGLVQPGRSLRLSCAASGFTFDDYAMHWVRQAPGKGLEWVSGISWNSGSIGYADSVKGRFTISRDNAKNSLYLQMNSLRAEDTALYYCAKDIWATVTPAAFDYWGQGTLVTVSS

SEQ ID NO: 76 - protein, 120 aa, synthetic construct
QVQLVQSGGGLVQPGRSLRLSCAASGFTFDDYAMHWVRQAPGKGLEWVSGISWNSGSIGYADSVKGRFTISRDNAKNSLYLQMNSLRAEDTALYYCAKDNSGSGRYFDYWGQGTLVTVSS

SEQ ID NO: 77 - protein, 121 aa, synthetic construct
QVQLVESGGGLVQPGRSLRLSCAASGFTFDDYAMHWVRQAPGKGLEWVSGISWNSGSIGYADSVKGRFTISRDNAKNSLYLQMNSLRAEDTALYYCAKDVTAMDTVGFQHWGQGTLVTVSS

SEQ ID NO: 78 - protein, 122 aa, synthetic construct
EVQLVQSGGGLVQPGRSLRLSCAASGFTFDDYAMHWVRQAPGKGLEWVSGISWNSGSIGYADSVKGRFTISRDNAKNSLYLQMNSLRAEDTALYYCAKGLVAATTPPYFDYWGQGTLVTVSS

SEQ ID NO: 79 - protein, 122 aa, synthetic construct
QVQLVQSGAEVKKPGSSVKVSCKASGGTFSSYAISWVRQAPGQGLEWMGGIIPIFGTANYAQKFQGRVTITADESTSTAYMELSSLRSEDTAVYYCARGTYYYDSSGTPDYWGQGTTVTVSS

SEQ ID NO: 80 - protein, 125 aa, synthetic construct
QVQLVQSGAEVKKPGSSVKVSCKASGGTFSSYAISWVRQAPGQGLEWMGGIIPIFGTANYAQKFQGRVTITADESTSTAYMELSSLRSEDTAVYYCARPSVLEWTYYYYYGMDVWGQGTLVTVSS

SEQ ID NO: 81 - protein, 113 aa, synthetic construct
QVQLVQSGAEVKKPGSSVKVSCKASGGTFSSYAISWVRQAPGQGLEWMGRIIPIFGIANYAQKFQGRVTITADKSTSTAYMELSSLRSEDTAVYYCARRFQHWGQGTLVTVSS

SEQ ID NO: 82 - protein, 121 aa, synthetic construct
EVQLLESGGGLVQPGGSLRLSCSASGFTFSSYAMHWVRQAPGKGLEYVSAISSNGGSTYYADSVKGRFTISRDNSKNTLYLQMSSLRAEDTAVYYCVKGEQWLAYNWFDPWGQGTTVTVSS

SEQ ID NO: 83 - protein, 121 aa, synthetic construct
QVQLVQSGGGVVQPGRSLRLSCAASGFTFSSYAMHWVRQAPGKGLEWVAVISYDGSNKYYADSVKGRFTISRDNSKNTLYLQMNSLRAEDTAVYYCARDSGPTTVTTFDYWGQGTLVTVSS

SEQ ID NO: 84 - protein, 119 aa, synthetic construct
QVQLVQSGGGVVQPGRSLRLSCAASGFTFSSYAMHWVRQAPGKGLEWVAVISYDGSNKYYADSVKGRFTISRDNSKNTLYLQMNSLRAEDTAVYYCARSVGYLNWFDPWGQGTLVTVSS

SEQ ID NO: 85 - protein, 125 aa, synthetic construct
QVQLVESGGGLVQPGGSLRLSCAASGFTFSSYAMSWVRQAPGKGLEWVSAISGSGGSTYYADSVKGRFTISRDNSKNTLYLQMNSLRAEDTAVYYCAKDHPPSVYSSSWLRFDYWGQGTTVTVSS

SEQ ID NO: 86 - protein, 128 aa, synthetic construct
EVQLVESGGGLVKPGGSLRLSCAASGFTFSSYAMSWVRQAPGKGLEWVSAISGSGGSTYYADSVKGRFTISRDNSKNTLYLQMNSLRAEDTAVYYCAKDLFLDLYDSSGYYLVPQIHWGQGTLVTVSS

SEQ ID NO: 87 - protein, 121 aa, synthetic construct
QVQLQESGGGVVQPGRSLRLSCAASGFTFSSYGMHWVRQAPGKGLEWVAVISYDGSNKYYADSVKGRFTISRDNSKNTLYLQMNSLRAEDTAVYYCATHGDYGGYQYFQHWGQGTTVTVSS

SEQ ID NO: 88 - protein, 123 aa, synthetic construct
QVQLVQSGGGLVKPGGSLRLSCAASGFTFSSYSMNWVRQAPGKGLEWVSSISSSSSYIYYADSVKGRFTISRDNAKNSLYLQMNSLRAEDTAVYYCARDRDTYYDYGDNFDYWGQGTLVTVSS

SEQ ID NO: 89 - protein, 115 aa, synthetic construct
QVQLVQSGGGLVQPGGSLRLSCAASGFTFSSYSMSWVRQAPGKGLEWVSAISGSGGTYYADSVKGRFTISRDSSKNTLYLQMNSLRAEDTAVYYCARSLRAFSYWGQGTLVTVSS

SEQ ID NO: 90 - protein, 123 aa, synthetic construct
QVQLVQSGAEVKKPGESLKISCKGSGYSFTSYWIGWVRQMPGKGLEWMGIIYPGDSDTRYSPSFQGQVTISADKSISTAYLQWSSLKASDTAMYYCARLGVSGSYRRSGMDVWGQGTLVTVSS

SEQ ID NO: 91 - protein, 110 aa, synthetic construct
QSALTQPASVSGSPGQSITISCTGTSSDVGGYNYVSWYQQHPGKAPKLMIYDVSNRPSGVSNRFSGSKSGNTASLTISGLQAEDEADYYCSSYTSSSTWVFGGGTKLTVL

SEQ ID NO: 92 - protein, 110 aa, synthetic construct
QSVLTQPPSVSGAPGQRVTISCTGSSSNIGAGYDVHWYQQLPGTAPKLLIYGNSNRPSGVPDRFSGSKSGTSASLAIAGLQAEDEADYYCQSYDSSLSVVFGGGTKVTVL

SEQ ID NO: 93 - protein, 111 aa, synthetic construct
DVVMTQSPLSLPVTPGEPASISCRSSQSLLHSNGYNYLDWYLQKPGQSPQLLIYLGSNRASGVPDRFSGSGSGTDFTLKISRVEAEDVGVYYCMQALQTPLFGPGTKVDIK

SEQ ID NO: 94 - protein, 111 aa, synthetic construct
QSALTQPASVSGSPGQSITISCTGTSSDVGGYNYVSWYQQHPGKAPKLMIYDVSNRPSGVSNRFSGSKSGNTASLTISGLQAEDEADYYCSSYTSSSTLVVFGGGTKLTVL

SEQ ID NO: 95 - protein, 112 aa, synthetic construct
DVVMTQSPLSLPVTPGEPASISCRSSQSLLHSNGYNYLDWYLQKPGQSPQLLIYLGSNRASGVPDRFSGSGSGTDFTLKISRVEAEDVGVYYCMQALQTPYTFGQGTKVDIK

SEQ ID NO: 96 - protein, 110 aa, synthetic construct
QSALTQPASVSGSPGQSITISCTGTSSDVGGYNYVSWYQQHPGKAPKLMIYDVSNRPSGVSNRFSGSKSGNTASLTISGLQAEDEADYYCSSYTSSSTLVFGGGTKVTVL

SEQ ID NO: 97 - protein, 110 aa, synthetic construct
QSVLTQPPSVSAAPGQKVTISCSGSSSNIGNNYVSWYQQLPGTAPKLLIYDNNKRPSGIPDRFSGSKSGTSATLGITGLQTGDEADYYCGTWDSSLSAVVFGGGTKLTVL

SEQ ID NO: 98 - protein, 107 aa, synthetic construct
DIQLTQSPSSLSASVGDRVTITCQASQDISNYLNWYQQKPGKAPKLLIYDASNLETGVPSRFSGSGSGTDFTFTISSLQPEDIATYYCQQYDNLPLTFGGGTKLEIK

SEQ ID NO: 99 - protein, 110 aa, synthetic construct
SYVLTQPPSASGTPGQRVTISCSGSSSNIGSNTVNWYQQLPGTAPKLLIYSNNQRPSGVPDRFSGSKSGTSASLAISGLQSEDEADYYCAAWDDSLNGYVFGTGTKLTVL

SEQ ID NO: 100 - protein, 112 aa, synthetic construct
QSVLTQPPSVSGAPGQRVTISCTGSSSNIGAGYDVHWYQQLPGTAPKLLIYGNSNRPSGVPDRFSGSKSGTSASLAITGLQAEDEADYYCQSYDSSLSGWGVFGGGTKLTVL

SEQ ID NO: 101 - protein, 111 aa, synthetic construct
QSVLTQPPSASGTPGQRVTISCSGSSSNIGSNYVYWYQQLPGTAPKLLIYRNSQRPSGVPDRFSGSKSGTSASLAISGLRSEDGADYYCAAWDDSLSVPYVFGTGTKLTVL

SEQ ID NO: 102 - protein, 107 aa, synthetic construct
DIQLTQSPSTLSASVGDRVTITCRASQSISSWLAWYQQKPGKAPKLLIYKASSLESGVPSRFSGSGSGTEFTLTISSLQPDDFATYYCQQYNSYLITFGQGTRLEIK

SEQ ID NO: 103 - protein, 112 aa, synthetic construct
QSVLTQPPSVSGAPGQRVTISCTGSSSNIGAGYDVHWYQQLPGTAPKLLIYGNSNRPSGVPDRFSGSKSGTSASLAITGLQAEDEADYYCQSYDSSLSGFVVFGGGTKLTVL

SEQ ID NO: 104 - protein, 110 aa, synthetic construct
QSALTQPASVSGSPGQSITISCTGTSSDVGGYNYVSWYQQHPGKAPKLMIYDVSNRPSGVSNRFSGSKSGNTASLTISGLQAEDEADYYCSSYTSSSTVVFGGGTKLTVL

SEQ ID NO: 105 - protein, 112 aa, synthetic construct
QSVLTQPPSVSGAPGQRVTISCTGSSSNIGAGYDVHWYQQLPGTAPKLLIYGNSNRPSGVPDRFSGSKSGTSASLAITGLQAEDEADYYCQSYDSSLSGSWVFGGGTKLTVL

SEQ ID NO: 106 - protein, 108 aa, synthetic construct
SYVLTQPPSVSVSPGQTARITCSGDALPKQYAYWYQQKPGQAPVLVIYKDSERPSGIPERFSGSSSGTTVTLTISGVQAEDEADYYCQSADSSGTYYVFGTGTKVTVL

SEQ ID NO: 107 - protein, 112 aa, synthetic construct
DVVMTQSPLSLPVTPGEPASISCRSSQSLLHSNGYNYLDWYLQKPGQSPQLLIYLGSNRASGVPDRFSGSGSGTDFTLNISRVEAEDVGVYYCMQSLRTPLTFGGGTKLEIK

SEQ ID NO: 108 - protein, 108 aa, synthetic construct
EIVLTQSPGTLSLSPGERATLSCRASQSVSSSYLAWYQQKPGQAPRLLIYGASSRATGIPDRFSGSGSGTDFTLTISRLEPEDFAVYYCQQYGSSPLTFGGGTKLEIK

SEQ ID NO: 109 - DNA, 366 bp, synthetic construct
  source 1..366: mol_type = other DNA
gaagtgcagcttgttcagagcgggggaggcctcgtccaacctggtcgatctttgaggctttcatgtgcagcttcaggttttacctttgacgactacgctatgcactgggttcgccaagctccaggtaagggtcttgaatgggtttcagggataagttggaactctggctccatcggctatgcagactcagtcaaaggcagattcaccatctcccgagataacgccaaaaatagtctctaccttcagatgaactctctcagggccgaggacactgcattgtattattgtgctaaaggccttgttgcggcaactacaccgccgtatttcgattactgggggcagggtacacttgtcactgtctcaagc

SEQ ID NO: 110 - DNA, 363 bp, synthetic construct
  source 1..363: mol_type = other DNA
caggttcagctggttcaaagcggcggcgggctcgtgcagccggggcgatcattgagactgtcctgtgcagcgtcaggttttacgttcgacgattatgccatgcactgggtccggcaagcaccaggaaaagggctcgagtgggtgtctggtatctcctggaactctggtagtatcggatatgcggacagtgtgaaagggcgattcacaatttcaagggataatgctaaaaacagcctctacttgcaaatgaacagcttgagagcagaagatacagccctgtactattgcgctaaggatatatctggctcacaactggttttgctggactactgggggcaaggcaccaccgtaacagtgagctct

SEQ ID NO: 111 - DNA, 360 bp, synthetic construct
  source 1..360: mol_type = other DNA
gaggttcaactgcttgagagtggaggtggtctggtacagccgggacgatccttgcgattgagctgtgcagccacaggattcacctttgacgattatgccatgcactgggtgagacaggcccctggaaaaggtttggagtgggttagcgggatcagttggaattccggctcaataggttatgccgattctgtaaagggacgctttacgatcagtagagacaatgccaaaaacagtctctacctgcaaatgaactcacttagggcagaggatacagccctgtattactgtgcgaaagcaaactactacgatagtagtgccctcgattattggggtcaaggaactctcgtcactgtcagcagc

SEQ ID NO: 112 - DNA, 363 bp, synthetic construct
  source 1..363: mol_type = other DNA
gaagtgcagcttctcgaaagcggagggggcctggtccaacctggtggctctctccgcctctcatgtagcgcctccggcttcaccttctcctcttatgcaatgcactgggtgcgccaggcacccggaaaaggcctcgaatacgttagcgctattagctccaacggaggaagcacatattacgctgacagtgtcaaaggacgctttaccataagccgcgataactccaagaataccctttatttgcaaatgagctcactccgggcagaggacaccgcagtgtactactgcgttaaaggagaacaatggttggcctacaattggtttgatccctggggtcaaggtactacggtgactgtttccagt

SEQ ID NO: 113 - DNA, 345 bp, synthetic construct
  source 1..345: mol_type = other DNA
caagtacaactcgtacaatccggaggaggcctggtacagcctggcggttcattgcggctctcctgtgcagcgtctggctttacgttctcatcctattctatgagttgggtccgccaagcgcctggcaaaggcttggagtgggtatcagcaatcagtggctctggtggaacatattatgcagattccgtgaaagggaggttcactatttcacgggattcttcaaaaaacacgttgtacctccaaatgaactctttgagggcagaagatactgccgtttattactgcgcgcgaagcctcagggcgttttcttactggggccaggggactttggttactgtctcttca

SEQ ID NO: 114 - DNA, 369 bp, synthetic construct
  source 1..369: mol_type = other DNA
caagttcaactcgtgcagtctggagcggaagttaaaaaaccaggggaatcactcaagatatcttgtaagggttctggttacagttttacctcatactggatagggtgggttcggcaaatgccaggcaagggactggagtggatgggcattatctatcctggagatagtgacactcgctacagcccatcttttcagggacaggtgacgatttccgccgataaaagcatctcaacggcgtaccttcagtggtctagcttgaaagccagcgatactgccatgtactattgcgcaaggctgggggtcagcggttcttaccgaagatcaggaatggacgtttggggtcaagggacccttgtaactgttagtagt

SEQ ID NO: 115 - DNA, 339 bp, synthetic construct
  source 1..339: mol_type = other DNA
caggtccaacttgtgcaaagcggtgccgaagttaagaagccggggtcatcagtgaaggtcagctgtaaagcgtctggtggaacattttctagctatgcgatctcatgggtgagacaggctccagggcagggcttggagtggatgggccgaatcatcccaatttttggaattgcgaactacgcacaaaagtttcaagggcgggtcaccattacagcagataaatcaacatcaacggcctacatggaactctcttccctgaggtctgaggacactgccgtttattattgtgctcgaagatttcaacactggggacaggggaccttggttacagtttcatca

SEQ ID NO: 116 - DNA, 360 bp, synthetic construct
  source 1..360: mol_type = other DNA
caggtacagttggtccagtcaggcgggggtcttgtgcaaccaggacgctcactccgcctttcctgcgcggcgtctggctttacgtttgatgattacgcaatgcactgggtaaggcaggccccaggtaaagggcttgaatgggtttcaggtatttcctggaatagcggaagtattggctacgcagactctgtgaaggggcggttcactatcagtcgggacaacgctaagaactccctgtacttgcagatgaattccctgagggcggaggatacagctctgtattattgtgctaaagacaactctggcagtggacgatattttgattactggggccaaggaactctcgtcacggttagtagc

SEQ ID NO: 117 - DNA, 330 bp, synthetic construct
  source 1..330: mol_type = other DNA
caatccgcacttacgcaaccggcgagcgtgagtggttcacctggacagagtatcactatttcctgtacggggaccagttcagatgttggcggatacaactacgtgtcatggtaccaacaacaccccgggaaagccccgaaattgatgatctatgatgtcagtaatcgcccttcaggtgtatccaacagattttcaggttctaaaagcggtaatacagcatcactcaccattagcgggctccaagccgaggacgaggcagattactactgctcctcatatacttcaagcagcactctggtgttcggcggagggactaaagtgactgttttg

SEQ ID NO: 118 - DNA, 330 bp, synthetic construct
  source 1..330: mol_type = other DNA
cagagtgtgttgactcaacctcccagcgttagtggggctccgggacaacgggttacgatcagttgtactggatcatcatccaacatcggcgccggttacgacgtgcattggtatcagcagctcccagggacggctcccaaacttctgatatacggtaatagtaataggccttcaggtgtacctgaccgcttctctggctccaaatcagggaccagtgcctctcttgctatcgcaggtttgcaagctgaggatgaagctgactattattgtcaaagttatgatagttccctttcagtcgtctttggtggcgggactaaggttacggtattg

SEQ ID NO: 119 - DNA, 360 bp, synthetic construct; identical to SEQ ID NO: 116
  source 1..360: mol_type = other DNA

SEQ ID NO: 120 - DNA, 336 bp, synthetic construct
  source 1..336: mol_type = other DNA
caaagcgtccttactcagcccccatctgtgtctggagcacctggtcaacgggttacaatatcatgtactggatcaagttcaaacataggcgccggatacgatgtgcattggtatcaacagttgccgggcacggcgccaaagttgcttatttatggtaactctaacagacctagcggcgttccagaccgcttctcaggcagcaagagcggcacaagtgcgagcctggcgataacgggactgcaagccgaggacgaagctgactactactgccaatcatatgattcatcactctcaggctggggggtatttgggggaggtacgaaactgactgtgctc

SEQ ID NO: 121 - DNA, 336 bp, synthetic construct
  source 1..336: mol_type = other DNA
gacgttgtcatgacgcagagtcccctctccctgccagttacacccggcgaacctgctagcattagttgcagaagttctcaatctcttctgcactctaatggatataattacctcgactggtatttgcaaaagccgggtcagagcccacagcttctcatatatctgggatctaaccgggcttctggagtccctgaccggttttccggttccggttctggtacggactttacccttaacatatcccgcgtagaagccgaagatgtgggagtctactactgtatgcaatcactgaggacccccctgaccttcggcggaggaactaaattggagatcaaa

SEQ ID NO: 122 - DNA, 324 bp, synthetic construct
  source 1..324: mol_type = other DNA
gagatcgtgttgacacaatccccggggacgttgtctctcagccctggagagcgggcaactctcagttgccgagcttctcagtccgtttccagtagctatctcgcctggtaccaacagaagccgggtcaagctccccggcttctgatttatggcgcatcatccagagctaccggcatcccggaccgattctctggctctggcagtggtactgattttacactgacgattagccggttggaaccagaggattttgccgtgtactactgccaacaatacggaagcagcccgcttacattcgggggaggtacaaaattggagatcaaa

SEQ ID NO: 123 - DNA, 330 bp, synthetic construct
  source 1..330: mol_type = other DNA
tcttacgttttgacccagcctcccagcgcgtcaggcacgcctggacagcgggtgaccatatcctgtagtggctctagtagcaatataggaagcaacacggtaaattggtatcaacagttgcccggaactgcacccaagctgttgatatatagcaataatcaaaggccgtctggagtacctgaccggttctcaggtagcaagagtgggacatctgcatcattggcgataagtggccttcagtcagaggatgaggctgactattattgtgcggcttgggacgactccttgaatggctatgtatttggcacggggaccaagctgacggtgctc

SEQ ID NO: 124 - DNA, 333 bp, synthetic construct
  source 1..333: mol_type = other DNA
cagagtgcgttgacacagcccgcatctgtgtctggttccccggggcagtctatcacaatttcatgcaccgggacctcctctgatgtcgggggatataattatgtaagttggtatcaacagcaccctggcaaggccccaaagctcatgatttatgacgtatcaaatagaccatctggagtgagtaacagatttagtggcagcaaaagtgggaacacggcttcccttacaatcagcgggttgcaagccgaggacgaagccgattactattgtagcagttacactagcagcagcaccctggtggtttttggggggggcaccaaattgacggtcctt

SEQ ID NO: 125 - protein, 330 aa, synthetic construct [sequence omitted]

SEQ ID NO: 126 - protein, 106 aa, synthetic construct
GQPKAAPSVTLFPPSSEELQANKATLVCLISDFYPGAVTVAWKADSSPVKAGVETTTPSKQSNNKYAASSYLSLTPEQWKSHRSYSCQVTHEGSTVEKTVAPTECS

SEQ ID NO: 127 - protein, 8 aa, synthetic construct
  VARIANT 6..7: note = X can be any amino acid
GCGCCXXC

SEQ ID NO: 128 - protein, 4 aa, synthetic construct
RFQH